European Patent Application EP 4 674 859 A1, published January 7, 2026. Title: METHOD FOR SCREENING TARGET MOLECULE CAPABLE OF FORMING COMPLEX WITH PLURAL KINDS OF TARGET MOLECULES AND METHOD FOR PRODUCING TARGET MOLECULE INCLUDING THE METHOD FOR SCREENING. Applicant: Chugai Pharmaceutical Co., Ltd. Application JP. The sequence listing filed with the application follows.

SEQUENCE LISTING (67 sequences)

SEQ ID NO: 1 - protein, 149 aa, synthetic construct
  SITE 144: note = Biotinylation
MGVQVETISPGDGRTFPKRGQTCVVHYTGMLEDGKKFDSSRDRNKPFKFMLGKQEVIRGWEEGVAQMSVGQRAKLTISPDYAYGATGHPGIIPPHATLVFDVELLKLEGGGSSDYKDDDDKSSGENLYFQSSGGGLNDIFEAQKIEWHE

SEQ ID NO: 2 - protein, 142 aa, synthetic construct
  SITE 137: note = Biotinylation
MELIRVAILWHEMWHEGLEEASRLYFGERNVKGMFEVLEPLHAMMERGPQTLKETSFNQAYGRDLMEAQEWCRKYMKSGNVKDLTQAWDLYYHVFRRISKQGGGSSDYKDDDDKSSGENLYFQSSGGGLNDIFEAQKIEWHE

SEQ ID NO: 3 - protein, 141 aa, synthetic construct
MGVQVETISPGDGRTFPKRGQTCVVHYTGMLEDGKKFDSSRDRNKPFKFMLGKQEVIRGWEEGVAQMSVGQRAKLTISPDYAYGATGHPGIIPPHATLVFDVELLKLEGGGSSDYKDDDDKGGSSLPMTGGGGSSHHHHHH

SEQ ID NO: 4 - protein, 134 aa, synthetic construct
MELIRVAILWHEMWHEGLEEASRLYFGERNVKGMFEVLEPLHAMMERGPQTLKETSFNQAYGRDLMEAQEWCRKYMKSGNVKDLTQAWDLYYHVFRRISKQGGGSSDYKDDDDKGGSSLPMTGGGGSSHHHHHH

SEQ ID NO: 5 - protein, 280 aa, synthetic construct
  SITE 11: note = Biotinylation
MGLNDIFEAQKIEWHESSGENLYFQSGGGSSDYKDDDDKSGGVQVETISPGDGRTFPKRGQTCVVHYTGMLEDGKKFDSSRDRNKPFKFMLGKQEVIRGWEEGVAQMSVGQRAKLTISPDYAYGATGHPGIIPPHATLVFDVELLKLEGSGSSGLEVLFQGPSSGSSGTELIRVAILWHEMWHEGLEEASRLYFGERNVKGMFEVLEPLHAMMERGPQTLKETSFNQAYGRDLMEAQEWCRKYMKSGNVKDLTQAWDLYYHVFRRISKQGGGSSHHHHHH

SEQ ID NO: 6 - protein, 206 aa, synthetic construct
  SITE 201: note = Biotinylation
GPMVNPTVFFDIAVDGEPLGRVSFELFADKVPKTAENFRALSTGEKGFGYKGSCFHRIIPGFMCQGGDFTRHNGTGGKSIYGEKFEDENFILKHTGPGILSMANAGPNTNGSQFFICTAKTEWLDGKHVVFGKVKEGMNIVEAMERFGSRNGKTSKKITIADCGQLEGSSDYKDDDDKSSGENLYFQSSGGGLNDIFEAQKIEWHE

SEQ ID NO: 7 - protein, 738 aa, synthetic construct
  SITE 733: note = Biotinylation
GPMGNEASYPLEMCSHFDADEIKRLGKRFKKLDLDNSGSLSVEEFMSLPELQQNPLVQRVIDIFDTDGNGEVDFKEFIEGVSQFSVKGDKEQKLRFAFRIYDMDKDGYISNGELFQVLKMMVGNNLKDTQLQQIVDKTIINADKDGDGRISFEEFCAVVGGLDIHKKMVVDVGGGGGGMSEPKAIDPKLSTTDRVVKAVPFPPSHRLTAKEVFDNDGKPRVDILKAHLMKEGRLEESVALRIITEGASILRQEKNLLDIDAPVTVCGDIHGQFFDLMKLFEVGGSPANTRYLFLGDYVDRGYFSIECVLYLWALKILYPKTLFLLRGNHECRHLTEYFTFKQECKIKYSERVYDACMDAFDCLPLAALMNQQFLCVHGGLSPEINTLDDIRKLDRFKEPPAYGPMCDILWSDPLEDFGNEKTQEHFTHNTVRGCSYFYSYPAVCEFLQHNNLLSILRAHEAQDAGYRMYRKSQTTGFPSLITIFSAPNYLDVYNNKAAVLKYENNVMNIRQFNCSPHPYWLPNFMDVFTWSLPFVGEKVTEMLVNVLNICSDDELGSEEDGFDGATAAARKEVIRNKIRAIGKMARVFSVLREESESVLTLKGLTPTGMLPSGVLSGGKQTLQSATVEAIEADEAIKGFSPQHKITSFEEAKGLDRINERMPPRRDAMPSDANLNSINKALTSETNGTDSNGSNSSNIQGSSDYKDDDDKSSGENLYFQSSGGGLNDIFEAQKIEWHE

SEQ ID NO: 8 - protein, 196 aa, synthetic construct
MVNPTVFFDIAVDGEPLGRVSFELFADKVPKTAENFRALSTGEKGFGYKGSCFHRIIPGFMCQGGDFTRHNGTGGKSIYGEKFEDENFILKHTGPGILSMANAGPNTNGSQFFICTAKTEWLDGKHVVFGKVKEGMNIVEAMERFGSRNGKTSKKITIADCGQLEGSSDYKDDDDKGGSSLPMTGGGGSSHHHHHH

SEQ ID NO: 9 - protein, 728 aa, synthetic construct
MGNEASYPLEMCSHFDADEIKRLGKRFKKLDLDNSGSLSVEEFMSLPELQQNPLVQRVIDIFDTDGNGEVDFKEFIEGVSQFSVKGDKEQKLRFAFRIYDMDKDGYISNGELFQVLKMMVGNNLKDTQLQQIVDKTIINADKDGDGRISFEEFCAVVGGLDIHKKMVVDVGGGGGGMSEPKAIDPKLSTTDRVVKAVPFPPSHRLTAKEVFDNDGKPRVDILKAHLMKEGRLEESVALRIITEGASILRQEKNLLDIDAPVTVCGDIHGQFFDLMKLFEVGGSPANTRYLFLGDYVDRGYFSIECVLYLWALKILYPKTLFLLRGNHECRHLTEYFTFKQECKIKYSERVYDACMDAFDCLPLAALMNQQFLCVHGGLSPEINTLDDIRKLDRFKEPPAYGPMCDILWSDPLEDFGNEKTQEHFTHNTVRGCSYFYSYPAVCEFLQHNNLLSILRAHEAQDAGYRMYRKSQTTGFPSLITIFSAPNYLDVYNNKAAVLKYENNVMNIRQFNCSPHPYWLPNFMDVFTWSLPFVGEKVTEMLVNVLNICSDDELGSEEDGFDGATAAARKEVIRNKIRAIGKMARVFSVLREESESVLTLKGLTPTGMLPSGVLSGGKQTLQSATVEAIEADEAIKGFSPQHKITSFEEAKGLDRINERMPPRRDAMPSDANLNSINKALTSETNGTDSNGSNSSNIQGSSDYKDDDDKGGSSLPMTGGGGSSHHHHHH

SEQ ID NO: 10 - protein, 920 aa, synthetic construct
  SITE 915: note = Biotinylation
MHHHHHHGNEASYPLEMCSHFDADEIKRLGKRFKKLDLDNSGSLSVEEFMSLPELQQNPLVQRVIDIFDTDGNGEVDFKEFIEGVSQFSVKGDKEQKLRFAFRIYDMDKDGYISNGELFQVLKMMVGNNLKDTQLQQIVDKTIINADKDGDGRISFEEFCAVVGGLDIHKKMVVDVGGGGGGSEPKAIDPKLSTTDRVVKAVPFPPSHRLTAKEVFDNDGKPRVDILKAHLMKEGRLEESVALRIITEGASILRQEKNLLDIDAPVTVCGDIHGQFFDLMKLFEVGGSPANTRYLFLGDYVDRGYFSIECVLYLWALKILYPKTLFLLRGNHECRHLTEYFTFKQECKIKYSERVYDACMDAFDCLPLAALMNQQFLCVHGGLSPEINTLDDIRKLDRFKEPPAYGPMCDILWSDPLEDFGNEKTQEHFTHNTVRGCSYFYSYPAVCEFLQHNNLLSILRAHEAQDAGYRMYRKSQTTGFPSLITIFSAPNYLDVYNNKAAVLKYENNVMNIRQFNCSPHPYWLPNFMDVFTWSLPFVGEKVTEMLVNVLNICSDDELGSEEDGFDGATAARAIGKMARVFSVLREESESVLTLKGLTPTGMLPSGVLSGGKQTLQSATVEAIEADEAIKGFSPQHKITSEEAKGLDRINERMPPRRDAMPSDANLNSINKALTSETNGTDSNGSNSSNIDGGGGSGLEVLFQGPGGGSGGGGSGGGSTVNPTVFFDIAVDGEPLGRVSFELFADKVPKTAENFRALSTGEKGFGYKGSCFHRIIPGFMCQGGDFTRHNGTGGKSIYGEKFEDENFILKHTGPGILSMANAGPNTNGSQFFICTAKTEWLDGKHVVFGKVKEGMNIVEAMERFGSRNGKTSKKITIADCGQLEDYKDDDDKGSGGENLYFQSSGGGLNDIFEAQKIEWHE

SEQ ID NO: 11 - DNA, 107 bp, synthetic construct
  source 1..107: mol_type = other DNA
  misc_feature 50..76: note = 9 repeats of the triplet randomly selected from the group consisting of TTT, TTG, CTT, CTG, ATT, ATG, GTT, GTG, TCT, TCG, CCG, ACT, GCT, TAC, CAT, CAG, AAC, GAT, GAG, TGC, TGG, CGT, CGG, AGT, AGG, and GGT.
gtaatacgactcactatagggttaactttaataaggagatataaatatgnnnnnnnnnnnnnnnnnnnnnnnnnnntagccgaccggcaccggcaccggcaaaaaaa

SEQ ID NO: 12 - DNA, 104 bp, synthetic construct
  source 1..104: mol_type = other DNA
  misc_feature 50..73: note = 8 repeats of the triplet randomly selected from the group consisting of TTT, TTG, CTT, CTG, ATT, ATG, GTT, GTG, TCT, TCG, CCG, ACT, GCT, TAC, CAT, CAG, AAC, GAT, GAG, TGC, TGG, CGT, CGG, AGT, AGG, and GGT.
gtaatacgactcactatagggttaactttaataaggagatataaatatgnnnnnnnnnnnnnnnnnnnnnnnntagccgaccggcaccggcaccggcaaaaaaa

SEQ ID NO: 13 - DNA, 38 bp, synthetic construct
  source 1..38: mol_type = other DNA
gtaatacgactcactatagggttaactttaataaggag

SEQ ID NO: 14 - DNA, 31 bp, synthetic construct
  source 1..31: mol_type = other DNA
tttttttgccggtgccggtgccggtcggcta

SEQ ID NO: 15 - DNA, 110 bp, synthetic construct
  source 1..110: mol_type = other DNA
ggcgtaatacgactcactatagggttaactttaataaggagatataaatatgcattcgggtgagtgccatactagttcttagccgaccggcaccggcaccggcaaaaaaa

SEQ ID NO: 16 - DNA, 110 bp, synthetic construct
  source 1..110: mol_type = other DNA
ggcgtaatacgactcactatagggttaactttaataaggagatataaatatgttttcggagtgcactaaccagccgttgtagccgaccggcaccggcaccggcaaaaaaa

SEQ ID NO: 17 - DNA, 110 bp, synthetic construct
  source 1..110: mol_type = other DNA
ggcgtaatacgactcactatagggttaactttaataaggagatataaatatgtctggtcgtcatctgtgccatattaggtagccgaccggcaccggcaccggcaaaaaaa

SEQ ID NO: 18 - DNA, 110 bp, synthetic construct
  source 1..110: mol_type = other DNA
ggcgtaatacgactcactatagggttaactttaataaggagatataaatatgtgggttttgctgtgctctactggtggttagccgaccggcaccggcaccggcaaaaaaa

SEQ ID NO: 19 - RNA, 89 nt, synthetic construct
  source 1..89: mol_type = other RNA
gggttaactttaataaggagatataaatatgcattcgggtgagtgccatactagttcttagccgaccggcaccggcaccggcaaaaaaa

SEQ ID NO: 20 - RNA, 89 nt, synthetic construct
  source 1..89: mol_type = other RNA
gggttaactttaataaggagatataaatatgttttcggagtgcactaaccagccgttgtagccgaccggcaccggcaccggcaaaaaaa

SEQ ID NO: 21 - RNA, 89 nt, synthetic construct
  source 1..89: mol_type = other RNA
gggttaactttaataaggagatataaatatgtctggtcgtcatctgtgccatattaggtagccgaccggcaccggcaccggcaaaaaaa

SEQ ID NO: 22 - RNA, 89 nt, synthetic construct
  source 1..89: mol_type = other RNA
gggttaactttaataaggagatataaatatgtgggttttgctgtgctctactggtggttagccgaccggcaccggcaccggcaaaaaaa

SEQ ID NO: 23 - DNA, 110 bp, synthetic construct
  source 1..110: mol_type = other DNA
ggcgtaatacgactcactatagggttaactttaataaggagatataaatatgcgtcagctgattcggtgggttgtgacttagccgaccggcaccggcaccggcaaaaaaa

SEQ ID NO: 24 - DNA, 110 bp, synthetic construct
  source 1..110: mol_type = other DNA
ggcgtaatacgactcactatagggttaactttaataaggagatataaatatgtggtttgataactcgaacgtggtgacttagccgaccggcaccggcaccggcaaaaaaa

SEQ ID NO: 25 - DNA, 110 bp, synthetic construct
  source 1..110: mol_type = other DNA
ggcgtaatacgactcactatagggttaactttaataaggagatataaatatgatgccgaggaacgttcttactactcagtagccgaccggcaccggcaccggcaaaaaaa

SEQ ID NO: 26 - DNA, 110 bp, synthetic construct
  source 1..110: mol_type = other DNA
ggcgtaatacgactcactatagggttaactttaataaggagatataaatatgtttagtggtattccgtgggttgtgatttagccgaccggcaccggcaccggcaaaaaaa

SEQ ID NO: 27 - RNA, 89 nt, synthetic construct
  source 1..89: mol_type = other RNA
gggttaactttaataaggagatataaatatgcgtcagctgattcggtgggttgtgacttagccgaccggcaccggcaccggcaaaaaaa

SEQ ID NO: 28 - RNA, 89 nt, synthetic construct
  source 1..89: mol_type = other RNA
gggttaactttaataaggagatataaatatgtggtttgataactcgaacgtggtgacttagccgaccggcaccggcaccggcaaaaaaa

SEQ ID NO: 29 - RNA, 89 nt, synthetic construct
  source 1..89: mol_type = other RNA
gggttaactttaataaggagatataaatatgatgccgaggaacgttcttactactcagtagccgaccggcaccggcaccggcaaaaaaa

SEQ ID NO: 30 - RNA, 89 nt, synthetic construct
  source 1..89: mol_type = other RNA
gggttaactttaataaggagatataaatatgtttagtggtattccgtgggttgtgatttagccgaccggcaccggcaccggcaaaaaaa

SEQ ID NO: 31 - DNA, 28 bp, synthetic construct
  source 1..28: mol_type = other DNA
  misc_feature 1: note = Substituent having an azide group is bound to phosphoric acid group.
tttttttgccggtgccggtgccggtcgg

SEQ ID NO: 32 - DNA, 110 bp, synthetic construct
  source 1..110: mol_type = other DNA
ggcgtaatacgactcactatagggttaactttaataaggagatataaatatggtttgctcttctaggtctctgaaccggtagccgaccggcaccggcaccggcaaaaaaa

SEQ ID NO: 33 - DNA, 110 bp, synthetic construct
  source 1..110: mol_type = other DNA
ggcgtaatacgactcactatagggttaactttaataaggagatataaatatgactctgaacgagtgcggtcattgccattagccgaccggcaccggcaccggcaaaaaaa

SEQ ID NO: 34 - DNA, 110 bp, synthetic construct
  source 1..110: mol_type = other DNA
ggcgtaatacgactcactatagggttaactttaataaggagatataaatatgcagttggagtggtttgtttggccgacttagccgaccggcaccggcaccggcaaaaaaa

SEQ ID NO: 35 - RNA, 89 nt, synthetic construct
  source 1..89: mol_type = other RNA
gggttaactttaataaggagatataaatatggtttgctcttctaggtctctgaaccggtagccgaccggcaccggcaccggcaaaaaaa

SEQ ID NO: 36 - RNA, 89 nt, synthetic construct
  source 1..89: mol_type = other RNA
gggttaactttaataaggagatataaatatgactctgaacgagtgcggtcattgccattagccgaccggcaccggcaccggcaaaaaaa

SEQ ID NO: 37 - RNA, 89 nt, synthetic construct
  source 1..89: mol_type = other RNA
gggttaactttaataaggagatataaatatgcagttggagtggtttgtttggccgacttagccgaccggcaccggcaccggcaaaaaaa

SEQ ID NO: 38 - DNA, 28 bp, synthetic construct
  source 1..28: mol_type = other DNA
tttttttgccggtgccggtgccggtcgg

SEQ ID NO: 39 - DNA, 110 bp, synthetic construct
  source 1..110: mol_type = other DNA
ggcgtaatacgactcactatagggttaactttaataaggagatataaatatgtctactgctgtgactaggttgaacagttagccgaccggcaccggcaccggcaaaaaaa

SEQ ID NO: 40 - DNA, 110 bp, synthetic construct
  source 1..110: mol_type = other DNA
ggcgtaatacgactcactatagggttaactttaataaggagatataaatatggattggccgggtttgcggactattggttagccgaccggcaccggcaccggcaaaaaaa

SEQ ID NO: 41 - DNA, 110 bp, synthetic construct
  source 1..110: mol_type = other DNA
ggcgtaatacgactcactatagggttaactttaataaggagatataaatatgatttgggttcttactaacactgttgtttagccgaccggcaccggcaccggcaaaaaaa

SEQ ID NO: 42 - RNA, 89 nt, synthetic construct
  source 1..89: mol_type = other RNA
gggttaactttaataaggagatataaatatgtctactgctgtgactaggttgaacagttagccgaccggcaccggcaccggcaaaaaaa

SEQ ID NO: 43 - RNA, 89 nt, synthetic construct
  source 1..89: mol_type = other RNA
gggttaactttaataaggagatataaatatggattggccgggtttgcggactattggttagccgaccggcaccggcaccggcaaaaaaa

SEQ ID NO: 44 - RNA, 89 nt, synthetic construct
  source 1..89: mol_type = other RNA
gggttaactttaataaggagatataaatatgatttgggttcttactaacactgttgtttagccgaccggcaccggcaccggcaaaaaaa

SEQ ID NO: 45 - protein, 9 aa, synthetic construct
PTGTGTGKK

SEQ ID NO: 46 - protein, 160 aa, synthetic construct
  SITE 155: note = Biotinylation
GLGGGGSGGGGSGVQVETISPGDGRTFPKRGQTCVVHYTGMLEDGKKFDSSRDRNKPFKFMLGKQEVIRGWEEGVAQMSVGQRAKLTISPDYAYGATGHPGIIPPHATLVFDVELLKLEGGGSSDYKDDDDKSSGENLYFQSSGGGLNDIFEAQKIEWHE

SEQ ID NO: 47 - protein, 328 aa, synthetic construct
ARDGDYLHLPSEVSRFFRPQETNDDHGEDSVGTRWAVLIAGSKGYANYRHQAGVCHAYQILKRGGLKDENIVVFMYDDIAYNESNPRPGVIINSPHGSDVYAGVPKDYTGEEVNAKNFLAAILGNKSAITGGSGKVVDSGPNDHIFIYYTDHGAAGVIGMPSKPYLYADELNDALKKKHASGTYKSLVFYLEACESGSMFEGILPEDLNIYALTSTNTTESSWAYYCPAQENPPPPEYNVCLGDLFSVAWLEDSDVQNSWYETLNQQYHHVDKRISHASHATQYGNLKLGEEGLFVYMGSNPANDNYTSLDGNALTPSSIVVNQRDAD

SEQ ID NO: 48 - protein, 156 aa, synthetic construct
MQAKPQIPKDKSKVAGYIEIPDADIKEPVYPGPATREQLNRGVSFAEENESLDDQNISIAGHTFIDRPNYQFTNLKAAKKGSMVYFKVGNETRKYKMTSIRNVKPTAVEVLDEQKGKDKQLTLITCDDYNEETGVWETRKIFVATEVKLEHHHHHH

SEQ ID NO: 49 - protein, 727 aa, synthetic construct
  SITE 727: note = N-{4-(4-methyltetrazinyl(phenlyacetyl)}lysine
MGNEASYPLEMCSHFDADEIKRLGKRFKKLDLDNSGSLSVEEFMSLPELQQNPLVQRVIDIFDTDGNGEVDFKEFIEGVSQFSVKGDKEQKLRFAFRIYDMDKDGYISNGELFQVLKMMVGNNLKDTQLQQIVDKTIINADKDGDGRISFEEFCAVVGGLDIHKKMVVDVGGGGGGMSEPKAIDPKLSTTDRVVKAVPFPPSHRLTAKEVFDNDGKPRVDILKAHLMKEGRLEESVALRIITEGASILRQEKNLLDIDAPVTVCGDIHGQFFDLMKLFEVGGSPANTRYLFLGDYVDRGYFSIECVLYLWALKILYPKTLFLLRGNHECRHLTEYFTFKQECKIKYSERVYDACMDAFDCLPLAALMNQQFLCVHGGLSPEINTLDDIRKLDRFKEPPAYGPMCDILWSDPLEDFGNEKTQEHFTHNTVRGCSYFYSYPAVCEFLQHNNLLSILRAHEAQDAGYRMYRKSQTTGFPSLITIFSAPNYLDVYNNKAAVLKYENNVMNIRQFNCSPHPYWLPNFMDVFTWSLPFVGEKVTEMLVNVLNICSDDELGSEEDGFDGATAAARKEVIRNKIRAIGKMARVFSVLREESESVLTLKGLTPTGMLPSGVLSGGKQTLQSATVEAIEADEAIKGFSPQHKITSFEEAKGLDRINERMPPRRDAMPSDANLNSINKALTSETNGTDSNGSNSSNIQGSSDYKDDDDKGGSSLPMTGGGGSGGGGSK

SEQ ID NO: 50 - protein, 174 aa, synthetic construct
  SITE 1: note = N-{(E)-cyclooct-4-enoxycarbonyl}glycine
  SITE 169: note = biotinylation
GGSGGGGSGGGGSNGLGGGGSGGGGSGVQVETISPGDGRTFPKRGQTCVVHYTGMLEDGKKFDSSRDRNKPFKFMLGKQEVIRGWEEGVAQMSVGQRAKLTISPDYAYGATGHPGIIPPHATLVFDVELLKLEGGGSSDYKDDDDKSSGENLYFQSSGGGLNDIFEAQKIEWHE

SEQ ID NO: 51 - DNA, 107 bp, synthetic construct
  source 1..107: mol_type = other DNA
gtaatacgactcactatagggttaactttaataaggagatataaatatgtgcacttctactggttactggcttcattagccgaccggcaccggcaccggcaaaaaaa

SEQ ID NO: 52 - DNA, 107 bp, synthetic construct
  source 1..107: mol_type = other DNA
gtaatacgactcactatagggttaactttaataaggagatataaatatgattaacgtgttttcgggttgctacccgtagccgaccggcaccggcaccggcaaaaaaa

SEQ ID NO: 53 - RNA, 89 nt, synthetic construct
  source 1..89: mol_type = other RNA
gggttaactttaataaggagatataaatatgtgcacttctactggttactggcttcattagccgaccggcaccggcaccggcaaaaaaa

SEQ ID NO: 54 - RNA, 89 nt, synthetic construct
  source 1..89: mol_type = other RNA
gggttaactttaataaggagatataaatatgattaacgtgttttcgggttgctacccgtagccgaccggcaccggcaccggcaaaaaaa

SEQ ID NO: 55 - protein, 311 aa, synthetic construct
  SITE 306: note = Biotinylation
MHHHHHHSGGVQVETISPGDGRTFPKRGQTCVVHYTGMLEDGKKFDSSRDRNKPFKFMLGKQEVIRGWEEGVAQMSVGQRAKLTISPDYAYGATGHPGIIPPHATLVFDVELLKLEGSGGGSGGGGSGGGGSGGGGSGGGGSGGGGSGGGGSGGGGSGGGGSGGGGSGGTELIRVAILWHEMWHEGLEEASRLYFGERNVKGMFEVLEPLHAMMERGPQTLKETSFNQAYGRDLMEAQEWCRKYMKSGNVKDLTQAWDLYYHVFRRISKQGGGSSDYKDDDDKSSGENLYFQSSGGGLNDIFEAQKIEWHE

SEQ ID NO: 56 - protein, 289 aa, synthetic construct
  SITE 11: note = Biotinylation
MGLNDIFEAQKIEWHESSGENLYFQSGGGSSDYKDDDDKSGGVQVETISPGDGRTFPKRGQTCVVHYTGMLEDGKKFDSSRDRNKPFKFMLGKQEVIRGWEEGVAQMSVGQRAKLTISPDYAYGATGHPGIIPPHATLVFDVELLKLEGSGSSGSSGLEVLFQGPSSGSSGSSGSSGTELIRVAILWHEMWHEGLEEASRLYFGERNVKGMFEVLEPLHAMMERGPQTLKETSFNQAYGRDLMEAQEWCRKYMKSGNVKDLTQAWDLYYHVFRRISKQGGGSSHHHHHH

SEQ ID NO: 57 - protein, 170 aa, synthetic construct
  SITE 23: note = Biotinylation
MDYKDDDDKGGSSGLNDIFEAQKIEWHESSGENLYFQGGGGSGVQVETISPGDGRTFPKRGQTCVVHYTGMLEDGKKFDSSRDRNKPFKFMLGKQEVIRGWEEGVAQMSVGQRAKLTISPDYAYGATGHPGIIPPHATLVFDVELLKLEGGGSSLPMTGGGGSSHHHHHH

SEQ ID NO: 58 - protein, 143 aa, synthetic construct
  SITE 11: note = Biotinylation
MGLNDIFEAQKIEWHESSGENLYFQGGGGSELIRVAILWHEMWHEGLEEASRLYFGERNVKGMFEVLEPLHAMMERGPQTLKETSFNQAYGRDLMEAQEWCRKYMKSGNVKDLTQAWDLYYHVFRRISKQGGGSSDYKDDDDK

SEQ ID NO: 59 - protein, 276 aa, synthetic construct
  SITE 23: note = Biotinylation
MDYKDDDDKGGSSGLNDIFEAQKIEWHESSGENLYFQGGGGSGVQVETISPGDGRTFPKRGQTCVVHYTGMLEDGKKFDSSRDRNKPFKFMLGKQEVIRGWEEGVAQMSVGQRAKLTISPDYAYGATGHPGIIPPHATLVFDVELLKLEGGGSSLPMTGGGGSELIRVAILWHEMWHEGLEEASRLYFGERNVKGMFEVLEPLHAMMERGPQTLKETSFNQAYGRDLMEAQEWCRKYMKSGNVKDLTQAWDLYYHVFRRISKQGGGSSDYKDDDDK

SEQ ID NO: 60 - protein, 125 aa, synthetic construct
GLGGGGSGGGGSELIRVAILWHEMWHEGLEEASRLYFGERNVKGMFEVLEPLHAMMERGPQTLKETSFNQAYGRDLMEAQEWCRKYMKSGNVKDLTQAWDLYYHVFRRISKQGGGSSDYKDDDDK

SEQ ID NO: 61 - protein, 307 aa, synthetic construct
  SITE 23: note = Biotinylation
MDYKDDDDKGGSSGLNDIFEAQKIEWHESSGENLYFQGGGGSGVQVETISPGDGRTFPKRGQTCVVHYTGMLEDGKKFDSSRDRNKPFKFMLGKQEVIRGWEEGVAQMSVGQRAKLTISPDYAYGATGHPGIIPPHATLVFDVELLKLEGGGSSLPMTGGGGGGGSGGGGSGGGGSGGGGSNGLGGGGSGGGGSELIRVAILWHEMWHEGLEEASRLYFGERNVKGMFEVLEPLHAMMERGPQTLKETSFNQAYGRDLMEAQEWCRKYMKSGNVKDLTQAWDLYYHVFRRISKQGGGSSDYKDDDDK

SEQ ID NO: 62 - protein, 27 aa, unidentified
GGGGGGGSGGGGSGGGGSGGGGSNGLH

SEQ ID NO: 63 - protein, 306 aa, synthetic construct
  SITE 301: note = Biotinylation
MELIRVAILWHEMWHEGLEEASRLYFGERNVKGMFEVLEPLHAMMERGPQTLKETSFNQAYGRDLMEAQEWCRKYMKSGNVKDLTQAWDLYYHVFRRISKQGGGSSDYKDDDDKGGSSLPMTGGGGGGGSGGGGSGGGGSGGGGSNGLGGGGSGGGGSGVQVETISPGDGRTFPKRGQTCVVHYTGMLEDGKKFDSSRDRNKPFKFMLGKQEVIRGWEEGVAQMSVGQRAKLTISPDYAYGATGHPGIIPPHATLVFDVELLKLEGGGSSDYKDDDDKSSGENLYFQSSGGGLNDIFEAQKIEWHE

SEQ ID NO: 64 - protein, 169 aa, synthetic construct
  SITE 169: note = N-{4-(4-methyltetrazinyl(phenlyacetyl)}lysine
  SITE 23: note = Biotinylation
MDYKDDDDKGGSSGLNDIFEAQKIEWHESSGENLYFQGGGGSGVQVETISPGDGRTFPKRGQTCVVHYTGMLEDGKKFDSSRDRNKPFKFMLGKQEVIRGWEEGVAQMSVGQRAKLTISPDYAYGATGHPGIIPPHATLVFDVELLKLEGGGSSLPMTGGGGSGGGGSK

SEQ ID NO: 65 - protein, 138 aa, synthetic construct
  SITE 138: note = N-{(E)-cyclooct-4-enoxycarbonyl}lycine
MELIRVAILWHEMWHEGLEEASRLYFGERNVKGMFEVLEPLHAMMERGPQTLKETSFNQAYGRDLMEAQEWCRKYMKSGNVKDLTQAWDLYYHVFRRISKQGGGSSDYKDDDDKGGSSLPMTGGGGSGGGGSGGGGSK

SEQ ID NO: 66 - protein, 174 aa, synthetic construct; identical to SEQ ID NO: 50
  SITE 1: note = N-{4-(4-methyltetrazinyl(phenlyacetyl)}glysine
  SITE 169: note = Biotinylation

SEQ ID NO: 67 - protein, 139 aa, synthetic construct
  SITE 1: note = N-{(E)-cyclooct-4-enoxycarbonyl}glycine
GGSGGGGSGGGGSNGLGGGGSGGGGSELIRVAILWHEMWHEGLEEASRLYFGERNVKGMFEVLEPLHAMMERGPQTLKETSFNQAYGRDLMEAQEWCRKYMKSGNVKDLTQAWDLYYHVFRRISKQGGGSSDYKDDDDK